European Patent Application EP 4 663 656 A2, published December 17, 2025. Title: MASP-2 AND MASP-3 INHIBITORS, AND RELATED COMPOSITIONS AND METHODS, FOR TREATMENT OF SICKLE CELL DISEASE. Applicant: Omeros Corporation. Application WO. The sequence listing filed with the application follows.

SEQUENCE LISTING (34 sequences)

SEQ ID NO: 1 - protein, 491 aa, synthetic construct
QVTLKESGPVLVKPTETLTLTCTVSGFSLSRGKMGVSWIRQPPGKALEWLAHIFSSDEKSYRTSLKSRLTISKDTSKNQVVLTMTNMDPVDTATYYCARIRRGGIDYWGQGTLVTVSSASTKGPSVFPLAPCSRSTSESTAALGCLVKDYFPEPVTVSWNSGALTSGVHTFPAVLQSSGLYSLSSVVTVPSSSLGTKTYTCNVDHKPSNTKVDKRVESKYGPPCPPCPAPEFLGGPSVFLFPPKPKDTLMISRTPEVTCVVVDVSQEDPEVQFNWYVDGVEVHNAKTKPREEQFNSTYRVVSVLTVLHQDWLNGKEYKCKVSNKGLPSSIEKTISKAKGQPREPQVYTLPPSQEEMTKNQVSLTCLVKGFYPSDIAVEWESNGQPENNYKTTPPVLDSDGSFFLYSRLTVDKSRWQEGNVFSCSVMHEALHNHYTQKSLSLSLGKAAGGSGLEVTCEPGTTFKDKCNTCRCGSDGKSAVCTKLWCNQGSGA

SEQ ID NO: 2 - protein, 36 aa, synthetic construct
LEVTCEPGTTFKDKCNTCRCGSDGKSAVCTKLWCNQ

SEQ ID NO: 3 - protein, 118 aa, synthetic construct
QVTLKESGPVLVKPTETLTLTCTVSGFSLSRGKMGVSWIRQPPGKALEWLAHIFSSDEKSYRTSLKSRLTISKDTSKNQVVLTMTNMDPVDTATYYCARIRRGGIDYWGQGTLVTVSS

SEQ ID NO: 4 - protein, 5 aa, synthetic construct
RGKMG

SEQ ID NO: 5 - protein, 16 aa, synthetic construct
LAHIFSSDEKSYRTSL

SEQ ID NO: 6 - protein, 13 aa, synthetic construct
YYCARIRRGGIDY

SEQ ID NO: 7 - protein, 106 aa, synthetic construct
QPVLTQPPSLSVSPGQTASITCSGEKLGDKYAYWYQQKPGQSPVLVMYQDKQRPSGIPERFSGSNSGNTATLTISGTQAMDEADYYCQAWDSSTAVFGGGTKLTVL

SEQ ID NO: 8 - protein, 11 aa, synthetic construct
GEKLGDKYAYW

SEQ ID NO: 9 - protein, 7 aa, synthetic construct
DKQRPSG

SEQ ID NO: 10 - protein, 9 aa, synthetic construct
AWDSSTAVF

SEQ ID NO: 11 - protein, 113 aa, synthetic construct
QVQLKQSGAELMKPGASVKLSCKATGYTFTGKWIEWVKQRPGHGLEWIGEILPGTGSTNYNEKFKGKATFTADSSSNTAYMQLSSLTTEDSAMYYCLRSEDVWGTGTTVTVSS

SEQ ID NO: 12 - protein, 5 aa, synthetic construct
GKWIE

SEQ ID NO: 13 - protein, 17 aa, synthetic construct
EILPGTGSTNYNEKFKG

SEQ ID NO: 14 - protein, 4 aa, synthetic construct
SEDV

SEQ ID NO: 15 - protein, 113 aa, synthetic construct
DIVMTQSPSSLAVSAGEKVTMSCKSSQSLLNSRTRKNYLAWYQQKPGQSPKLLIYWASTRESGVPDRFTGSGSGTDFTLTISSVQAEDLAVYYCKQSYNIPTFGGGTKLEIKR

SEQ ID NO: 16 - protein, 17 aa, synthetic construct
KSSQSLLNSRTRKNYLA

SEQ ID NO: 17 - protein, 7 aa, synthetic construct
WASTRES

SEQ ID NO: 18 - protein, 8 aa, synthetic construct
KQSYNIPT

SEQ ID NO: 19 - protein, 121 aa, synthetic construct
QVQLVQSGAEVKKPGASVKVSCKASGYTFTNHHMHWLRQAPGQGLEWIGDIDASDSETHYIEKFKDRATLTIDKSSSTAYMELSSLRSEDTAVYYCARGDITTTLRYFDVWGQGTLVTVSS

SEQ ID NO: 20 - protein, 5 aa, synthetic construct
NHHMH

SEQ ID NO: 21 - protein, 17 aa, synthetic construct
DIDASDSETHYIEKFKD

SEQ ID NO: 22 - protein, 12 aa, synthetic construct
GDITTTLRYFDV

SEQ ID NO: 23 - protein, 107 aa, synthetic construct
DIQLTQSPSSLSASVGDRVTITCSASSSVRYMYWYQQKPGKAPKLLIYDTSNLASGVPSRFSGSGSGTDNTLTISSLQPEDFATYYCQQWSSYPLTFGQGTKVEIKR

SEQ ID NO: 24 - protein, 10 aa, synthetic construct
SASSSVRYMY

SEQ ID NO: 25 - protein, 7 aa, synthetic construct
DTSNLAS

SEQ ID NO: 26 - protein, 9 aa, synthetic construct
QQWSSYPLT

SEQ ID NO: 27 - protein, 121 aa, synthetic construct
QVQLQQPGAELVRPGSSVRLSCKASGYTFTNYWMHWLKQRPIQGLEWIGDIDPSDSETHYIEKFKDKATLTIDKSSSTAYMHLSSLTSEDSAIYYCARGDITTTLRYFDVWGTGTTVTVSS

SEQ ID NO: 28 - protein, 5 aa, synthetic construct
NYWMH

SEQ ID NO: 29 - protein, 17 aa, synthetic construct
DIDPSDSETHYIEKFKD

SEQ ID NO: 30 - protein, 107 aa, synthetic construct
QIVLTQSPVIMSASPGEKVTMTCSASSSVRYMYWYQQKPGSSPRLLIYDTSNLASGVPVRFSGSGSGTSNSLTISRMEAEDAATYYCQQWSSYPLTFGAGTKLELKR

SEQ ID NO: 31 - protein, 121 aa, synthetic construct
QVQLVQSGAEVKKPGASVKVSCKASGYTFTNYWMHWLRQAPGQGLEWIGDIDPSDSETHYIEKFKDRATLTIDKSSSTAYMELSSLRSEDTAVYYCARGDITTTLRYFDVWGQGTLVTVSS

SEQ ID NO: 32 - protein, 121 aa, synthetic construct
QVQLVQSGAEVKKPGASVKVSCKASGYTFTNYWMHWLRQAPGQGLEWIGDIDASDSETHYIEKFKDRATLTIDKSSSTAYMELSSLRSEDTAVYYCARGDITTTLRYFDVWGQGTLVTVSS

SEQ ID NO: 33 - protein, 121 aa, synthetic construct
QVQLVQSGAEVKKPGASVKVSCKASGYTFTNYHMHWLRQAPGQGLEWIGDIDASDSETHYIEKFKDRATLTIDKSSSTAYMELSSLRSEDTAVYYCARGDITTTLRYFDVWGQGTLVTVSS

SEQ ID NO: 34 - protein, 5 aa, synthetic construct
NYHMH